European Patent Specification EP 3 544 990 B1, published July 2, 2025. Title: Viral Vector Constructs for Expression of Genetic Adjuvants Activating the CD40 and STING Pathways. Applicant: aratinga.bio AIO. Application PCT/IB2017/001553. The sequence listing filed with the application follows.

SEQUENCE LISTING (24 sequences)

SEQ ID NO: 1 - DNA, 1158 bp, Epstein Barr virus
atggatctggacctggaaagaggacctcctggacctagacggcctcctagaggaccacctctgagcagctctattggactggccctgctgctgcttctgctggctctgctgttctggctgtacatcatcatgagcaactggaccggcggagcactgctggtgctgtatgcctttgctctgatgctggtcatcatcatcctgatcatcttcatcttccggcgggacctgctgtgtcctctgggagcactttgtctgttgctgctgatgatcaccctcctgctgatcgccctgtggaacctgcatggacaggccctgtatctgggaatcgtgctgttcatcttcggctgcctgctggttctcggcctgtggatctacctgctggaaatcctttggagactgggcgccaccatctggcagctgctggcctttttcctggccttctttctggatatcatcctcctcatcattgccctgtacctgcagcagaactggtggaccctgctggtggatctgctttggctgctgctctttctggccatcctgatttggatgtactaccacggccagcggcacagcgacgaacaccaccatgatgacagcctgcctcatcctcagcaggccaccgacgatagcagcaaccagagcgacagcaacagcaacgagggcagacatctgctgctggtgtctggtgctggcgacggacctcctctgtgttctcaaaatcttggcgcccctggcggcggaccaaacaatggacctcaggaccccgacaacaccgacgacaatggccctcaagatcctgataataccgatgacaacggcccacacgaccctctgcctcaagacccagataacacagacgataacggtccacaagatccggacaatactgacgataatggaccccacgatccactgcctcacaaccctagcgatagcgccggaaatgatggcggacctccacagctgaccgaggaagtggaaaacaaaggcggagatcagggccctcctctgatgaccgatggcggaggtggacactctcacgattctggccacgacggcatcgaccctcatctgcctacactgctgctcggcacatctggctctggcggcgacgatgatgatcctcatggacctgtgcagctgagctactacgac

SEQ ID NO: 2 - protein, 386 aa, Epstein Barr virus
MDLDLERGPPGPRRPPRGPPLSSSIGLALLLLLLALLFWLYIIMSNWTGGALLVLYAFALMLVIIILIIFIFRRDLLCPLGALCLLLLMITLLLIALWNLHGQALYLGIVLFIFGCLLVLGLWIYLLEILWRLGATIWQLLAFFLAFFLDIILLIIALYLQQNWWTLLVDLLWLLLFLAILIWMYYHGQRHSDEHHHDDSLPHPQQATDDSSNQSDSNSNEGRHLLLVSGAGDGPPLCSQNLGAPGGGPNNGPQDPDNTDDNGPQDPDNTDDNGPHDPLPQDPDNTDDNGPQDPDNTDDNGPHDPLPHNPSDSAGNDGGPPQLTEEVENKGGDQGPPLMTDGGGGHSHDSGHDGIDPHLPTLLLGTSGSGGDDDDPHGPVQLSYYD

SEQ ID NO: 3 - DNA, 570 bp, Epstein Barr virus
atggatctggatctcgaaagaggacctcctggacctagacggcctcctagaggaccacctctgagcagctctattggactggccctgctgctgcttctgctggctctgctgttctggctgtacatcatcatgagcaactggaccggcggagcactgctggtgctgtatgcctttgctctgatgctggtcatcatcatcctgatcatcttcatcttccggcgggacctgctgtgtcctctgggagcactttgtctgttgctgctgatgatcaccctcctgctgatcgccctgtggaacctgcatggacaggccctgtatctgggcatcgtgctgttcatcttcggctgcctgctggttctcggcctgtggatctacctgctggaaatcctttggagactgggcgccaccatctggcagctgctggcctttttcctggccttctttctggatatcatcctcctcatcattgccctgtacctgcagcagaactggtggaccctgctggtggatctgctttggctgctgctctttctggccatcctgatttggatgtactaccacggccagcgg

SEQ ID NO: 4 - protein, 190 aa, Epstein Barr virus
MDLDLERGPPGPRRPPRGPPLSSSIGLALLLLLLALLFWLYIIMSNWTGGALLVLYAFALMLVIIILIIFIFRRDLLCPLGALCLLLLMITLLLIALWNLHGQALYLGIVLFIFGCLLVLGLWIYLLEILWRLGATIWQLLAFFLAFFLDIILLIIALYLQQNWWTLLVDLLWLLLFLAILIWMYYHGQR

SEQ ID NO: 5 - DNA, 2187 bp, Artificial sequence
  Fusion of LMP-1 from Epstein Barr virus and ISP1 from Homo sapiens
atggatctggatctcgaaagaggacctcctggacctagacggcctcctagaggaccacctctgagcagctctattggactggccctgctgctgcttctgctggctctgctgttctggctgtacatcatcatgagcaactggaccggcggagcactgctggtgctgtatgcctttgctctgatgctggtcatcatcatcctgatcatcttcatcttccggcgggacctgctgtgtcctctgggagcactttgtctgttgctgctgatgatcaccctcctgctgatcgccctgtggaacctgcatggacaggccctgtatctgggcatcgtgctgttcatcttcggctgcctgctggttctcggcctgtggatctacctgctggaaatcctttggagactgggcgccaccatctggcagctgctggcctttttcctggccttctttctggatatcatcctcctcatcattgccctgtacctgcagcagaactggtggaccctgctggtggatctgctttggctgctgctctttctggccatcctgatttggatgtactaccacggccagcggcctttcgccgaggacaagacctacaagtacatctgccggaacttcagcaacttctgcaacgtggacgtggtggaaattctgccctacctgccttgcctgaccgccagagatcaggacagactgagagccacatgtaccctgagcggcaacagagacacactgtggcacctgttcaacaccctgcagagaaggcctggctgggtcgagtactttatcgccgctctgagaggctgcgagctggtcgatctggctgatgaagtggccagcgtgtaccagagctaccagcctagaaccagcgaccggcctcctgatcctctcgaacctccatctctgcccgccgaaagacctggacctcctacaccagctgccgctcacagcatcccttacaacagctgcagagagaaagaacctagctaccccatgcctgtgcaagagacacaggccccagaaagccctggcgagaatagcgaacaggctctgcagacactgagccccagagccattcctagaaaccctgatggcggccctctggaaagctctagtgatctggccgctctgtcccctctgacaagctctggacaccaagagcaggataccgagctgggcagcacacatacagccggcgctacaagcagcctgacaccttctagaggccccgtgtctcccagcgtgtcatttcagcctctggccaggtctacccctagggcttctagactgcctggaccaacaggcagcgtggtgtctaccggcacaagcttcagctctagctctcctggactggctagtgccggtgccgctgagggaaaacaaggcgccgaatctgatcaggccgagcctatcatctgtagcagcggagcagaagcccctgccaatagcctgcctagcaaggtgccaaccacactgatgcccgtgaacacagtggccctgaaggtgccagctaatcctgcctccgtgtccaccgtgccttctaagctgccaaccagctctaagccacctggcgccgtgccatctaacgccctgacaaatcctgctccaagcaagctgcccatcaactccacaagagccggcatggtgccctctaaggtgcccacatctatggtgctgaccaaggtgtccgccagcaccgtgccaacagatggcagctccagaaacgaggaaacccctgccgctcctactcctgctggcgctacaggcggatcttctgcttggctggatagcagcagcgagaacagaggcctgggcagcgagctttctaaacctggcgtgctggcttcccaggtggacagcccattttccggctgctttgaggacctggctatcagcgcctctacaagcctcggcatgggaccttgtcacggccccgaggaaaacgagtacaagagcgagggcaccttcggcatccacgtggccgagaatcctagcatccaactgctggaaggcaaccccggacctccagctgatccagatggcggaccaagacctcaggccgacagaaagttccaagagcgcgaggtgccctgccacagaccttctccaggtgctctgtggctgcaggttgcagtgacaggcgtcctggtggttacactgctcgtggtcctgtatagacggcggctgcac

SEQ ID NO: 6 - protein, 729 aa, Artificial sequence
  Fusion of LMP1 from Epstein Barr virus and ISP1 from Homo sapiens
MDLDLERGPPGPRRPPRGPPLSSSIGLALLLLLLALLFWLYIIMSNWTGGALLVLYAFALMLVIIILIIFIFRRDLLCPLGALCLLLLMITLLLIALWNLHGQALYLGIVLFIFGCLLVLGLWIYLLEILWRLGATIWQLLAFFLAFFLDIILLIIALYLQQNWWTLLVDLLWLLLFLAILIWMYYHGQRPFAEDKTYKYICRNFSNFCNVDVVEILPYLPCLTARDQDRLRATCTLSGNRDTLWHLFNTLQRRPGWVEYFIAALRGCELVDLADEVASVYQSYQPRTSDRPPDPLEPPSLPAERPGPPTPAAAHSIPYNSCREKEPSYPMPVQETQAPESPGENSEQALQTLSPRAIPRNPDGGPLESSSDLAALSPLTSSGHQEQDTELGSTHTAGATSSLTPSRGPVSPSVSFQPLARSTPRASRLPGPTGSVVSTGTSFSSSSPGLASAGAAEGKQGAESDQAEPIICSSGAEAPANSLPSKVPTTLMPVNTVALKVPANPASVSTVPSKLPTSSKPPGAVPSNALTNPAPSKLPINSTRAGMVPSKVPTSMVLTKVSASTVPTDGSSRNEETPAAPTPAGATGGSSAWLDSSSENRGLGSELSKPGVLASQVDSPFSGCFEDLAISASTSLGMGPCHGPEENEYKSEGTFGIHVAENPSIQLLEGNPGPPADPDGGPRPQADRKFQEREVPCHRPSPGALWLQVAVTGVLVVTLLVVLYRRRLH

SEQ ID NO: 7 - DNA, 2106 bp, Artificial sequence
  Fusion of LMP1 from Epstein Barr virus and IPS1 from Homo sapiens
atggatctggatctcgaaagaggacctcctggacctagacggcctcctagaggaccacctctgagcagctctattggactggccctgctgctgcttctgctggctctgctgttctggctgtacatcatcatgagcaactggaccggcggagcactgctggtgctgtatgcctttgctctgatgctggtcatcatcatcctgatcatcttcatcttccggcgggacctgctgtgtcctctgggagcactttgtctgttgctgctgatgatcaccctcctgctgatcgccctgtggaacctgcatggacaggccctgtatctgggcatcgtgctgttcatcttcggctgcctgctggttctcggcctgtggatctacctgctggaaatcctttggagactgggcgccaccatctggcagctgctggcctttttcctggccttctttctggatatcatcctcctcatcattgccctgtacctgcagcagaactggtggaccctgctggtggatctgctttggctgctgctctttctggccatcctgatttggatgtactaccacggccagcggcctttcgccgaggacaagacctacaagtacatctgccggaacttcagcaacttctgcaacgtggacgtggtggaaattctgccctacctgccttgcctgaccgccagagatcaggacagactgagagccacatgtaccctgagcggcaacagagacacactgtggcacctgttcaacaccctgcagagaaggcctggctgggtcgagtactttatcgccgctctgagaggctgcgagctggtcgatctggctgatgaagtggccagcgtgtaccagagctaccagcctagaaccagcgaccggcctcctgatcctctcgaacctccatctctgcccgccgaaagacctggacctcctacaccagctgccgctcacagcatcccttacaacagctgcagagagaaagaacctagctaccccatgcctgtgcaagagacacaggccccagaaagccctggcgagaatagcgaacaggctctgcagacactgagccccagagccattcctagaaaccctgatggcggccctctggaaagctctagtgatctggccgctctgtcccctctgacaagctctggacaccaagagcaggataccgagctgggcagcacacatacagccggcgctacaagcagcctgacaccttctagaggccccgtgtctcccagcgtgtcatttcagcctctggccaggtctacccctagggcttctagactgcctggaccaacaggcagcgtggtgtctaccggcacaagcttcagctctagctctcctggactggctagtgccggtgccgctgagggaaaacaaggcgccgaatctgatcaggccgagcctatcatctgtagcagcggagcagaagcccctgccaatagcctgcctagcaaggtgccaaccacactgatgcccgtgaacacagtggccctgaaggtgccagctaatcctgcctccgtgtccaccgtgccttctaagctgccaaccagctctaagccacctggcgccgtgccatctaacgccctgacaaatcctgctccaagcaagctgcccatcaactccacaagagccggcatggtgccctctaaggtgcccacatctatggtgctgaccaaggtgtccgccagcaccgtgccaacagatggcagctccagaaacgaggaaacccctgccgctcctactcctgctggcgctacaggcggatcttctgcttggctggatagcagcagcgagaacagaggcctgggcagcgagctttctaaacctggcgtgctggcttcccaggtggacagcccattttccggctgctttgaggacctggctatcagcgcctctacaagcctcggcatgggaccttgtcacggccccgaggaaaacgagtacaagagcgagggcaccttcggcatccacgtggccgagaatcctagcatccaactgctggaaggcaaccccggacctccagctgatccagatggcggaccaagacctcaggccgacagaaagttccaagagcgcgaggtgccctgccacagaccttctcca

SEQ ID NO: 8 - protein, 702 aa, Artificial sequence
  Fusion of LMP1 from Epstein Barr virus and IPS1 from Homo sapiens
MDLDLERGPPGPRRPPRGPPLSSSIGLALLLLLLALLFWLYIIMSNWTGGALLVLYAFALMLVIIILIIFIFRRDLLCPLGALCLLLLMITLLLIALWNLHGQALYLGIVLFIFGCLLVLGLWIYLLEILWRLGATIWQLLAFFLAFFLDIILLIIALYLQQNWWTLLVDLLWLLLFLAILIWMYYHGQRPFAEDKTYKYICRNFSNFCNVDVVEILPYLPCLTARDQDRLRATCTLSGNRDTLWHLFNTLQRRPGWVEYFIAALRGCELVDLADEVASVYQSYQPRTSDRPPDPLEPPSLPAERPGPPTPAAAHSIPYNSCREKEPSYPMPVQETQAPESPGENSEQALQTLSPRAIPRNPDGGPLESSSDLAALSPLTSSGHQEQDTELGSTHTAGATSSLTPSRGPVSPSVSFQPLARSTPRASRLPGPTGSVVSTGTSFSSSSPGLASAGAAEGKQGAESDQAEPIICSSGAEAPANSLPSKVPTTLMPVNTVALKVPANPASVSTVPSKLPTSSKPPGAVPSNALTNPAPSKLPINSTRAGMVPSKVPTSMVLTKVSASTVPTDGSSRNEETPAAPTPAGATGGSSAWLDSSSENRGLGSELSKPGVLASQVDSPFSGCFEDLAISASTSLGMGPCHGPEENEYKSEGTFGIHVAENPSIQLLEGNPGPPADPDGGPRPQADRKFQEREVPCHRPSP

SEQ ID NO: 9 - DNA, 1953 bp, Artificial sequence
  Fusion of LMP1 of Epstein Barr virus and IPS1 from Homo sapiens
atggatctggatctcgaaagaggacctcctggacctagacggcctcctagaggaccacctctgagcagctctattggactggccctgctgctgcttctgctggctctgctgttctggctgtacatcatcatgagcaactggaccggcggagcactgctggtgctgtatgcctttgctctgatgctggtcatcatcatcctgatcatcttcatcttccggcgggacctgctgtgtcctctgggagcactttgtctgttgctgctgatgatcaccctcctgctgatcgccctgtggaacctgcatggacaggccctgtatctgggcatcgtgctgttcatcttcggctgcctgctggttctcggcctgtggatctacctgctggaaatcctttggagactgggcgccaccatctggcagctgctggcctttttcctggccttctttctggatatcatcctcctcatcattgccctgtacctgcagcagaactggtggaccctgctggtggatctgctttggctgctgctctttctggccatcctgatttggatgtactaccacggccagcggcctttcgccgaggacaagacctacaagtacatctgccggaacttcagcaacttctgcaacgtggacgtggtggaaattctgccctacctgccttgcctgaccgccagagatcaggacagactgagagccacatgtaccctgagcggcaacagagacacactgtggcacctgttcaacaccctgcagagaaggcctggctgggtcgagtactttatcgccgctctgagaggctgcgagctggtcgatctggctgatgaagtggccagcgtgtaccagagctaccagcctagaaccagcgaccggggcgagaatagcgaacaggctctgcagacactgagccccagagccattcctagaaaccctgatggcggccctctggaaagctctagtgatctggccgctctgtcccctctgacaagctctggacaccaagagcaggataccgagctgggcagcacacatacagccggcgctacaagcagcctgacaccttctagaggccccgtgtctcccagcgtgtcatttcagcctctggccaggtctacccctagggcttctagactgcctggaccaacaggcagcgtggtgtctaccggcacaagcttcagctctagctctcctggactggctagtgccggtgccgctgagggaaaacaaggcgccgaatctgatcaggccgagcctatcatctgtagcagcggagcagaagcccctgccaatagcctgcctagcaaggtgccaaccacactgatgcccgtgaacacagtggccctgaaggtgccagctaatcctgcctccgtgtccaccgtgccttctaagctgccaaccagctctaagccacctggcgccgtgccatctaacgccctgacaaatcctgctccaagcaagctgcccatcaactccacaagagccggcatggtgccctctaaggtgcccacatctatggtgctgaccaaggtgtccgccagcaccgtgccaacagatggcagctccagaaacgaggaaacccctgccgctcctactcctgctggcgctacaggcggatcttctgcttggctggatagcagcagcgagaacagaggcctgggcagcgagctttctaaacctggcgtgctggcttcccaggtggacagcccattttccggctgctttgaggacctggctatcagcgcctctacaagcctcggcatgggaccttgtcacggccccgaggaaaacgagtacaagagcgagggcaccttcggcatccacgtggccgagaatcctagcatccaactgctggaaggcaaccccggacctccagctgatccagatggcggaccaagacctcaggccgacagaaagttccaagagcgcgaggtgccctgccacagaccttctcca

SEQ ID NO: 10 - protein, 651 aa, Artificial Sequence
  Fustion of LMP1 of Epstein Barr virus and IPS1 of Homo sapiens
MDLDLERGPPGPRRPPRGPPLSSSIGLALLLLLLALLFWLYIIMSNWTGGALLVLYAFALMLVIIILIIFIFRRDLLCPLGALCLLLLMITLLLIALWNLHGQALYLGIVLFIFGCLLVLGLWIYLLEILWRLGATIWQLLAFFLAFFLDIILLIIALYLQQNWWTLLVDLLWLLLFLAILIWMYYHGQRPFAEDKTYKYICRNFSNFCNVDVVEILPYLPCLTARDQDRLRATCTLSGNRDTLWHLFNTLQRRPGWVEYFIAALRGCELVDLADEVASVYQSYQPRTSDRGENSEQALQTLSPRAIPRNPDGGPLESSSDLAALSPLTSSGHQEQDTELGSTHTAGATSSLTPSRGPVSPSVSFQPLARSTPRASRLPGPTGSVVSTGTSFSSSSPGLASAGAAEGKQGAESDQAEPIICSSGAEAPANSLPSKVPTTLMPVNTVALKVPANPASVSTVPSKLPTSSKPPGAVPSNALTNPAPSKLPINSTRAGMVPSKVPTSMVLTKVSASTVPTDGSSRNEETPAAPTPAGATGGSSAWLDSSSENRGLGSELSKPGVLASQVDSPFSGCFEDLAISASTSLGMGPCHGPEENEYKSEGTFGIHVAENPSIQLLEGNPGPPADPDGGPRPQADRKFQEREVPCHRPSP

SEQ ID NO: 11 - DNA, 2109 bp, Artificial sequence
  Fustion of LMP1 of Epstein Barr virus and IPS1 of Homo sapiens
atggatctggatctcgaaagaggacctcctggacctagacggcctcctagaggaccacctctgagcagctctattggactggccctgctgctgcttctgctggctctgctgttctggctgtacatcatcatgagcaactggaccggcggagcactgctggtgctgtatgcctttgctctgatgctggtcatcatcatcctgatcatcttcatcttccggcgggacctgctgtgtcctctgggagcactttgtctgttgctgctgatgatcaccctcctgctgatcgccctgtggaacctgcatggacaggccctgtatctgggcatcgtgctgttcatcttcggctgcctgctggttctcggcctgtggatctacctgctggaaatcctttggagactgggcgccaccatctggcagctgctggcctttttcctggccttctttctggatatcatcctcctcatcattgccctgtacctgcagcagaactggtggaccctgctggtggatctgctttggctgctgctctttctggccatcctgatttggatgtactaccacggccagcggcccagccccagacactgccccgtggagagagagcagttcaagagagacgcccagcccagacccggcggcgaccccgacgccccccccggccccaacggcgagctgctgcagatcagccccaacgaggccgtgcacatcggcttcaccggcgagagcaagtacgagaacgaggagcccggccactgccccggcatgggcctgagcaccagcgccagcatcgccctggacgagttctgcggcagcttccccagcgacgtgcagagcgccctggtgggccccaagagcctggagagcggcctgggcagaaacgagagcagcagcgacctgtgggccagcagcggcggcaccgccggcgcccccacccccgccgcccccaccgaggagaacagaagcagcggcgacacccccgtgaccagcgccagcgtgaagaccctggtgatgagcacccccgtgaagagccccgtgatgggcgccagaaccagcaacatccccctgaagagccccgcccccaacaccctggccaacagccccgtggccggcccccccaagagcagcacccccctgaagagccccgtgaccagcgtgagcgcccccaacgcccccgtgaagctggccgtgaccaacgtgcccatgctgaccacccccgtgaagagccccctgagcaacgcccccgccgaggccggcagcagctgcatcatccccgaggcccaggacagcgaggccggccagaagggcgaggccgccggcgccagcgccctgggccccagcagcagcagcttcagcaccggcaccagcgtggtgagcggcacccccggccccctgagaagcgccagacccaccagcagagccctgccccagttcagcgtgagccccagcgtgcccggcagaagccccaccctgagcagcaccgccggcgccacccacaccagcggcctggagaccgaccaggagcagcacggcagcagcaccctgcccagcctggccgccctggacagcagcagcgagctgcccggcggcgaccccaacagacccatcgccagacccagcctgacccagctggcccaggagagcaacgagggccccagcgagcccgcccagaccgagcaggtgcccatgccctacagccccgagaaggagagatgcagcaactaccccatcagccacgccgccgcccccaccccccccggccccagagaggcccccctgagcccccccgagctgcccgacccccccagagacagcaccagaccccagtacagccagtacgtgagcgccgtggaggacgccctggacgtgctggagtgcggcagactggccgccatcttctacgaggtgtggggccccagaagacagctgaccaacttcctgcactggctgaccgacagaaacggcagcctgacctgcaccgccagactgagagaccaggacagagccaccctgtgccccctgtaccccctgatcgaggtggtggacgtgaactgcttcaacagcttcaacagatgcatctacaagtacaccaaggacgaggccttccccatg

SEQ ID NO: 12 - protein, 703 aa, Artificial sequence
  Fusion of LMP1 of Epstein Barr Virus and IPS1 of Homo sapiens
MDLDLERGPPGPRRPPRGPPLSSSIGLALLLLLLALLFWLYIIMSNWTGGALLVLYAFALMLVIIILIIFIFRRDLLCPLGALCLLLLMITLLLIALWNLHGQALYLGIVLFIFGCLLVLGLWIYLLEILWRLGATIWQLLAFFLAFFLDIILLIIALYLQQNWWTLLVDLLWLLLFLAILIWMYYHGQRPSPRHCPVEREQFKRDAQPRPGGDPDAPPGPNGELLQISPNEAVHIGFTGESKYENEEPGHCPGMGLSTSASIALDEFCGSFPSDVQSALVGPKSLESGLGRNESSSDLWASSGGTAGAPTPAAPTEENRSSGDTPVTSASVKTLVMSTPVKSPVMGARTSNIPLKSPAPNTLANSPVAGPPKSSTPLKSPVTSVSAPNAPVKLAVTNVPMLTTPVKSPLSNAPAEAGSSCIIPEAQDSEAGQKGEAAGASALGPSSSSFSTGTSVVSGTPGPLRSARPTSRALPQFSVSPSVPGRSPTLSSTAGATHTSGLETDQEQHGSSTLPSLAALDSSSELPGGDPNRPIARPSLTQLAQESNEGPSEPAQTEQVPMPYSPEKERCSNYPISHAAAPTPPGPREAPLSPPELPDPPRDSTRPQYSQYVSAVEDALDVLECGRLAAIFYEVWGPRRQLTNFLHWLTDRNGSLTCTARLRDQDRATLCPLYPLIEVVDVNCFNSFNRCIYKYTKDEAFPM

SEQ ID NO: 13 - DNA, 2694 bp, Artificial sequence
  Fusion of LMP1 of Epstein Barr virus and IPS1 of Homo sapiens
atggatctggacctggaaagaggacctcctggacctagacggcctcctagaggaccacctctgagcagctctattggactggccctgctgctgcttctgctggctctgctgttctggctgtacatcatcatgagcaactggaccggcggagcactgctggtgctgtatgcctttgctctgatgctggtcatcatcatcctgatcatcttcatcttccggcgggacctgctgtgtcctctgggagcactttgtctgttgctgctgatgatcaccctcctgctgatcgccctgtggaacctgcatggacaggccctgtatctgggaatcgtgctgttcatcttcggctgcctgctggttctcggcctgtggatctacctgctggaaatcctttggagactgggcgccaccatctggcagctgctggcctttttcctggccttctttctggatatcatcctcctcatcattgccctgtacctgcagcagaactggtggaccctgctggtggatctgctttggctgctgctctttctggccatcctgatttggatgtactaccacggccagcggcacagcgacgaacaccaccatgatgacagcctgcctcatcctcagcaggccaccgacgatagcagcaaccagagcgacagcaacagcaacgagggcagacatctgctgctggtgtctggtgctggcgacggacctcctctgtgttctcaaaatcttggcgcccctggcggcggaccaaacaatggacctcaggaccccgacaacaccgacgacaatggccctcaagatcctgataataccgatgacaacggcccacacgaccctctgcctcaagacccagataacacagacgataacggtccacaagatccggacaatactgacgataatggaccccacgatccactgcctcacaaccctagcgatagcgccggaaatgatggcggacctccacagctgaccgaggaagtggaaaacaaaggcggagatcagggccctcctctgatgaccgatggcggaggtggacactctcacgattctggccacgacggcatcgaccctcatctgcctacactgctgctcggcacatctggctctggcggcgacgatgatgatcctcatggacctgtgcagctgagctactacgaccctttcgccgaggacaagacctacaagtacatctgccggaacttcagcaacttctgcaacgtggacgtggtggaaattctgccctacctgccttgcctgaccgccagagatcaggacagactgagagccacatgtaccctgagcggcaacagagacacactgtggcacctgttcaacaccctgcagagaaggcctggctgggtcgagtactttatcgccgctctgagaggctgcgagctggtcgatctggctgatgaagtggccagcgtgtaccagagctaccagcctagaaccagcgaccggcctcctgatcctctcgaacctccatctctgcccgccgaaagacctggacctcctacaccagctgccgctcacagcatcccttacaacagctgcagagagaaagaacctagctaccccatgcctgtgcaagagacacaggccccagaaagccctggcgagaatagcgaacaggctctgcagacactgagccccagagccattcctagaaaccctgatggcggccctctggaaagctctagtgatctggccgctctgtcccctctgacaagctctggacaccaagagcaggataccgagctgggcagcacacatacagccggcgctacaagcagcctgacaccttctagaggccccgtgtctcccagcgtgtcatttcagcctctggccaggtctacccctagggcttctagactgcctggaccaacaggcagcgtggtgtctaccggcacaagcttcagctctagctctcctggactggctagtgccggtgccgctgagggaaaacaaggcgccgaatctgatcaggccgagcctatcatctgtagcagcggagcagaagcccctgccaatagcctgcctagcaaggtgccaaccacactgatgcccgtgaacacagtggccctgaaggtgccagctaatcctgcctccgtgtccaccgtgccttctaagctgccaaccagctctaagccacctggcgccgtgccatctaacgccctgacaaatcctgctccaagcaagctgcccatcaactccacaagagccggcatggtgccctctaaggtgcccacatctatggtgctgaccaaggtgtccgccagcaccgtgccaacagatggcagctccagaaacgaggaaacccctgccgctcctactcctgctggcgctacaggcggatcttctgcttggctggatagcagcagcgagaacagaggcctgggcagcgagctttctaaacctggcgtgctggcttcccaggtggacagcccattttccggctgctttgaggacctggctatcagcgcctctacaagcctcggcatgggaccttgtcacggccccgaggaaaacgagtacaagagcgagggcaccttcggcatccacgtggccgagaatcctagcatccaactgctggaaggcaaccccggacctccagctgatccagatggcggaccaagacctcaggccgacagaaagttccaagagcgcgaggtgccctgccacagaccttctcca

SEQ ID NO: 14 - protein, 898 aa, Artificial sequence
  Fusion of LMP1 of Epstein Barr virus and IPS1 of Homo sapiens
MDLDLERGPPGPRRPPRGPPLSSSIGLALLLLLLALLFWLYIIMSNWTGGALLVLYAFALMLVIIILIIFIFRRDLLCPLGALCLLLLMITLLLIALWNLHGQALYLGIVLFIFGCLLVLGLWIYLLEILWRLGATIWQLLAFFLAFFLDIILLIIALYLQQNWWTLLVDLLWLLLFLAILIWMYYHGQRHSDEHHHDDSLPHPQQATDDSSNQSDSNSNEGRHLLLVSGAGDGPPLCSQNLGAPGGGPNNGPQDPDNTDDNGPQDPDNTDDNGPHDPLPQDPDNTDDNGPQDPDNTDDNGPHDPLPHNPSDSAGNDGGPPQLTEEVENKGGDQGPPLMTDGGGGHSHDSGHDGIDPHLPTLLLGTSGSGGDDDDPHGPVQLSYYDPFAEDKTYKYICRNFSNFCNVDVVEILPYLPCLTARDQDRLRATCTLSGNRDTLWHLFNTLQRRPGWVEYFIAALRGCELVDLADEVASVYQSYQPRTSDRPPDPLEPPSLPAERPGPPTPAAAHSIPYNSCREKEPSYPMPVQETQAPESPGENSEQALQTLSPRAIPRNPDGGPLESSSDLAALSPLTSSGHQEQDTELGSTHTAGATSSLTPSRGPVSPSVSFQPLARSTPRASRLPGPTGSVVSTGTSFSSSSPGLASAGAAEGKQGAESDQAEPIICSSGAEAPANSLPSKVPTTLMPVNTVALKVPANPASVSTVPSKLPTSSKPPGAVPSNALTNPAPSKLPINSTRAGMVPSKVPTSMVLTKVSASTVPTDGSSRNEETPAAPTPAGATGGSSAWLDSSSENRGLGSELSKPGVLASQVDSPFSGCFEDLAISASTSLGMGPCHGPEENEYKSEGTFGIHVAENPSIQLLEGNPGPPADPDGGPRPQADRKFQEREVPCHRPSP

SEQ ID NO: 15 - DNA, 2541 bp, Artificial sequence
  LMP1 of Epstein Barr virus and IPS1 of Homo sapiens
atggatctggacctggaaagaggacctcctggacctagacggcctcctagaggaccacctctgagcagctctattggactggccctgctgctgcttctgctggctctgctgttctggctgtacatcatcatgagcaactggaccggcggagcactgctggtgctgtatgcctttgctctgatgctggtcatcatcatcctgatcatcttcatcttccggcgggacctgctgtgtcctctgggagcactttgtctgttgctgctgatgatcaccctcctgctgatcgccctgtggaacctgcatggacaggccctgtatctgggaatcgtgctgttcatcttcggctgcctgctggttctcggcctgtggatctacctgctggaaatcctttggagactgggcgccaccatctggcagctgctggcctttttcctggccttctttctggatatcatcctcctcatcattgccctgtacctgcagcagaactggtggaccctgctggtggatctgctttggctgctgctctttctggccatcctgatttggatgtactaccacggccagcggcacagcgacgaacaccaccatgatgacagcctgcctcatcctcagcaggccaccgacgatagcagcaaccagagcgacagcaacagcaacgagggcagacatctgctgctggtgtctggtgctggcgacggacctcctctgtgttctcaaaatcttggcgcccctggcggcggaccaaacaatggacctcaggaccccgacaacaccgacgacaatggccctcaagatcctgataataccgatgacaacggcccacacgaccctctgcctcaagacccagataacacagacgataacggtccacaagatccggacaatactgacgataatggaccccacgatccactgcctcacaaccctagcgatagcgccggaaatgatggcggacctccacagctgaccgaggaagtggaaaacaaaggcggagatcagggccctcctctgatgaccgatggcggaggtggacactctcacgattctggccacgacggcatcgaccctcatctgcctacactgctgctcggcacatctggctctggcggcgacgatgatgatcctcatggacctgtgcagctgagctactacgaccctttcgccgaggacaagacctacaagtacatctgccggaacttcagcaacttctgcaacgtggacgtggtggaaattctgccctacctgccttgcctgaccgccagagatcaggacagactgagagccacatgtaccctgagcggcaacagagacacactgtggcacctgttcaacaccctgcagagaaggcctggctgggtcgagtactttatcgccgctctgagaggctgcgagctggtcgatctggctgatgaagtggccagcgtgtaccagagctaccagcctagaaccagcgaccggggcgagaatagcgaacaggctctgcagacactgagccccagagccattcctagaaaccctgatggcggccctctggaaagctctagtgatctggccgctctgtcccctctgacaagctctggacaccaagagcaggataccgagctgggcagcacacatacagccggcgctacaagcagcctgacaccttctagaggccccgtgtctcccagcgtgtcatttcagcctctggccaggtctacccctagggcttctagactgcctggaccaacaggcagcgtggtgtctaccggcacaagcttcagctctagctctcctggactggctagtgccggtgccgctgagggaaaacaaggcgccgaatctgatcaggccgagcctatcatctgtagcagcggagcagaagcccctgccaatagcctgcctagcaaggtgccaaccacactgatgcccgtgaacacagtggccctgaaggtgccagctaatcctgcctccgtgtccaccgtgccttctaagctgccaaccagctctaagccacctggcgccgtgccatctaacgccctgacaaatcctgctccaagcaagctgcccatcaactccacaagagccggcatggtgccctctaaggtgcccacatctatggtgctgaccaaggtgtccgccagcaccgtgccaacagatggcagctccagaaacgaggaaacccctgccgctcctactcctgctggcgctacaggcggatcttctgcttggctggatagcagcagcgagaacagaggcctgggcagcgagctttctaaacctggcgtgctggcttcccaggtggacagcccattttccggctgctttgaggacctggctatcagcgcctctacaagcctcggcatgggaccttgtcacggccccgaggaaaacgagtacaagagcgagggcaccttcggcatccacgtggccgagaatcctagcatccaactgctggaaggcaaccccggacctccagctgatccagatggcggaccaagacctcaggccgacagaaagttccaagagcgcgaggtgccctgccacagaccttctcca

SEQ ID NO: 16 - protein, 847 aa, Artificial sequence
  Fusion of LMP1 of Epstein Barr virus and IPS1 of Homo sapiens
MDLDLERGPPGPRRPPRGPPLSSSIGLALLLLLLALLFWLYIIMSNWTGGALLVLYAFALMLVIIILIIFIFRRDLLCPLGALCLLLLMITLLLIALWNLHGQALYLGIVLFIFGCLLVLGLWIYLLEILWRLGATIWQLLAFFLAFFLDIILLIIALYLQQNWWTLLVDLLWLLLFLAILIWMYYHGQRHSDEHHHDDSLPHPQQATDDSSNQSDSNSNEGRHLLLVSGAGDGPPLCSQNLGAPGGGPNNGPQDPDNTDDNGPQDPDNTDDNGPHDPLPQDPDNTDDNGPQDPDNTDDNGPHDPLPHNPSDSAGNDGGPPQLTEEVENKGGDQGPPLMTDGGGGHSHDSGHDGIDPHLPTLLLGTSGSGGDDDDPHGPVQLSYYDPFAEDKTYKYICRNFSNFCNVDVVEILPYLPCLTARDQDRLRATCTLSGNRDTLWHLFNTLQRRPGWVEYFIAALRGCELVDLADEVASVYQSYQPRTSDRGENSEQALQTLSPRAIPRNPDGGPLESSSDLAALSPLTSSGHQEQDTELGSTHTAGATSSLTPSRGPVSPSVSFQPLARSTPRASRLPGPTGSVVSTGTSFSSSSPGLASAGAAEGKQGAESDQAEPIICSSGAEAPANSLPSKVPTTLMPVNTVALKVPANPASVSTVPSKLPTSSKPPGAVPSNALTNPAPSKLPINSTRAGMVPSKVPTSMVLTKVSASTVPTDGSSRNEETPAAPTPAGATGGSSAWLDSSSENRGLGSELSKPGVLASQVDSPFSGCFEDLAISASTSLGMGPCHGPEENEYKSEGTFGIHVAENPSIQLLEGNPGPPADPDGGPRPQADRKFQEREVPCHRPSP

SEQ ID NO: 17 - DNA, 2697 bp, Artificial sequence
  Fusion of LMP1 of Epstein Barr virus and IPS1 of Homo sapiens
atggatctggacctggaaagaggacctcctggacctagacggcctcctagaggaccacctctgagcagctctattggactggccctgctgctgcttctgctggctctgctgttctggctgtacatcatcatgagcaactggaccggcggagcactgctggtgctgtatgcctttgctctgatgctggtcatcatcatcctgatcatcttcatcttccggcgggacctgctgtgtcctctgggagcactttgtctgttgctgctgatgatcaccctcctgctgatcgccctgtggaacctgcatggacaggccctgtatctgggaatcgtgctgttcatcttcggctgcctgctggttctcggcctgtggatctacctgctggaaatcctttggagactgggcgccaccatctggcagctgctggcctttttcctggccttctttctggatatcatcctcctcatcattgccctgtacctgcagcagaactggtggaccctgctggtggatctgctttggctgctgctctttctggccatcctgatttggatgtactaccacggccagcggcacagcgacgaacaccaccatgatgacagcctgcctcatcctcagcaggccaccgacgatagcagcaaccagagcgacagcaacagcaacgagggcagacatctgctgctggtgtctggtgctggcgacggacctcctctgtgttctcaaaatcttggcgcccctggcggcggaccaaacaatggacctcaggaccccgacaacaccgacgacaatggccctcaagatcctgataataccgatgacaacggcccacacgaccctctgcctcaagacccagataacacagacgataacggtccacaagatccggacaatactgacgataatggaccccacgatccactgcctcacaaccctagcgatagcgccggaaatgatggcggacctccacagctgaccgaggaagtggaaaacaaaggcggagatcagggccctcctctgatgaccgatggcggaggtggacactctcacgattctggccacgacggcatcgaccctcatctgcctacactgctgctcggcacatctggctctggcggcgacgatgatgatcctcatggacctgtgcagctgagctactacgacccttctccaagacactgcccagtggaaagagagcagttcaagagggacgcccagcctagacctggcggagatcctgatgctccacctggaccaaatggcgagctgctgcagatcagccctaatgaggccgtgcacatcggcttcaccggcgagtctaagtacgagaacgaggaacccggccactgtcctggcatgggcctttctacatctgcctctatcgccctggacgagttctgcggcagctttccatctgatgtgcagtctgccctcgtgggccctaagtctctggaatctggcctgggcagaaacgagagcagctccgatctgtgggctagctctggtggaacagctggcgctcctacaccagccgctcctaccgaagagaatagaagcagcggcgacacccctgtgacaagcgcctctgtgaaaaccctggtcatgagcaccccagtgaagtccccagtgatgggcgccagaacctccaacattcccctgaagtctcccgctcctaacacactggccaactctccagtggctggccctcctaagtctagcacccctctgaaaagccccgtgacctctgtgtctgcccctaacgctcctgtgaaactggccgtgaccaacgtgcccatgctgaccacacctgtgaaatccccactgagcaatgcccctgccgaggccggaagctcttgtatcattcccgaggctcaggatagcgaggctggccaaaaaggcgaagctgcaggcgcttctgctctgggccctagctctagctcttttagcaccggcaccagcgtggtgtctggcacaccaggacctctgagaagcgccagacctacctctagagccctgcctcagtttagcgtgtcccctagtgtgcctggcagaagccctacactgtctagtacagccggcgctacacacaccagcggactggaaacagaccaagaacagcatggcagcagcaccctgccttctctggctgcccttgattctagcagcgaactgccaggcggcgaccccaatagacctatcgctagacctagcctgacacagctggcccaagagagcaatgagggcccttctgagcctgctcagaccgaacaggtgccaatgccttacagccccgagaaagagcggtgcagcaactaccctatcagccatgccgctgctcccacacctcctggtccaagagaagctcctctgagccctcctgagctgcccgatcctccaagagatagcaccagacctcagtactcccagtacgtgtccgccgtggaagatgccctggatgtgctggaatgtggcagactggccgccatcttctacgaagtgtggggccctagaaggcagctgaccaactttctgcactggctgaccgacagaaacggcagcctgacatgtaccgccagactgagagatcaggaccgggccacactgtgccctctgtatcctctgatcgaggtggtggacgtgaactgcttcaacagcttcaaccggtgcatctacaagtacaccaaggacgaggctttccctatg

SEQ ID NO: 18 - protein, 899 aa, Artificial sequence
  Fusion of LMP1 of Epstein Barr virus and IPS1 of Homo sapiens
MDLDLERGPPGPRRPPRGPPLSSSIGLALLLLLLALLFWLYIIMSNWTGGALLVLYAFALMLVIIILIIFIFRRDLLCPLGALCLLLLMITLLLIALWNLHGQALYLGIVLFIFGCLLVLGLWIYLLEILWRLGATIWQLLAFFLAFFLDIILLIIALYLQQNWWTLLVDLLWLLLFLAILIWMYYHGQRHSDEHHHDDSLPHPQQATDDSSNQSDSNSNEGRHLLLVSGAGDGPPLCSQNLGAPGGGPNNGPQDPDNTDDNGPQDPDNTDDNGPHDPLPQDPDNTDDNGPQDPDNTDDNGPHDPLPHNPSDSAGNDGGPPQLTEEVENKGGDQGPPLMTDGGGGHSHDSGHDGIDPHLPTLLLGTSGSGGDDDDPHGPVQLSYYDPSPRHCPVEREQFKRDAQPRPGGDPDAPPGPNGELLQISPNEAVHIGFTGESKYENEEPGHCPGMGLSTSASIALDEFCGSFPSDVQSALVGPKSLESGLGRNESSSDLWASSGGTAGAPTPAAPTEENRSSGDTPVTSASVKTLVMSTPVKSPVMGARTSNIPLKSPAPNTLANSPVAGPPKSSTPLKSPVTSVSAPNAPVKLAVTNVPMLTTPVKSPLSNAPAEAGSSCIIPEAQDSEAGQKGEAAGASALGPSSSSFSTGTSVVSGTPGPLRSARPTSRALPQFSVSPSVPGRSPTLSSTAGATHTSGLETDQEQHGSSTLPSLAALDSSSELPGGDPNRPIARPSLTQLAQESNEGPSEPAQTEQVPMPYSPEKERCSNYPISHAAAPTPPGPREAPLSPPELPDPPRDSTRPQYSQYVSAVEDALDVLECGRLAAIFYEVWGPRRQLTNFLHWLTDRNGSLTCTARLRDQDRATLCPLYPLIEVVDVNCFNSFNRCIYKYTKDEAFPM

SEQ ID NO: 19 - DNA, 2694 bp, Artificial sequence
  Fusion of LMP1 of Epstein Barr virus and IPS1 of Homo sapiens
atggatctggatctcgaaagaggacctcctggacctagacggcctcctagaggaccacctctgagcagctctattggactggccctgctgctgcttctgctggctctgctgttctggctgtacatcatcatgagcaactggaccggcggagcactgctggtgctgtatgcctttgctctgatgctggtcatcatcatcctgatcatcttcatcttccggcgggacctgctgtgtcctctgggagcactttgtctgttgctgctgatgatcaccctcctgctgatcgccctgtggaacctgcatggacaggccctgtatctgggcatcgtgctgttcatcttcggctgcctgctggttctcggcctgtggatctacctgctggaaatcctttggagactgggcgccaccatctggcagctgctggcctttttcctggccttctttctggatatcatcctcctcatcattgccctgtacctgcagcagaactggtggaccctgctggtggatctgctttggctgctgctctttctggccatcctgatttggatgtactaccacggccagcggcctttcgccgaggacaagacctacaagtacatctgccggaacttcagcaacttctgcaacgtggacgtggtggaaattctgccctacctgccttgcctgaccgccagagatcaggacagactgagagccacatgtaccctgagcggcaacagagacacactgtggcacctgttcaacaccctgcagagaaggcctggctgggtcgagtactttatcgccgctctgagaggctgcgagctggtcgatctggctgatgaagtggccagcgtgtaccagagctaccagcctagaaccagcgaccggcctcctgatcctctcgaacctccatctctgcccgccgaaagacctggacctcctacaccagctgccgctcacagcatcccttacaacagctgcagagagaaagaacctagctaccccatgcctgtgcaagagacacaggccccagaaagccctggcgagaatagcgaacaggctctgcagacactgagccccagagccattcctagaaaccctgatggcggccctctggaaagctctagtgatctggccgctctgtcccctctgacaagctctggacaccaagagcaggataccgagctgggcagcacacatacagccggcgctacaagcagcctgacaccttctagaggccccgtgtctcccagcgtgtcatttcagcctctggccaggtctacccctagggcttctagactgcctggaccaacaggcagcgtggtgtctaccggcacaagcttcagctctagctctcctggactggctagtgccggtgccgctgagggaaaacaaggcgccgaatctgatcaggccgagcctatcatctgtagcagcggagcagaagcccctgccaatagcctgcctagcaaggtgccaaccacactgatgcccgtgaacacagtggccctgaaggtgccagctaatcctgcctccgtgtccaccgtgccttctaagctgccaaccagctctaagccacctggcgccgtgccatctaacgccctgacaaatcctgctccaagcaagctgcccatcaactccacaagagccggcatggtgccctctaaggtgcccacatctatggtgctgaccaaggtgtccgccagcaccgtgccaacagatggcagctccagaaacgaggaaacccctgccgctcctactcctgctggcgctacaggcggatcttctgcttggctggatagcagcagcgagaacagaggcctgggcagcgagctttctaaacctggcgtgctggcttcccaggtggacagcccattttccggctgctttgaggacctggctatcagcgcctctacaagcctcggcatgggaccttgtcacggccccgaggaaaacgagtacaagagcgagggcaccttcggcatccacgtggccgagaatcctagcatccaactgctggaaggcaaccccggacctccagctgatccagatggcggaccaagacctcaggccgacagaaagttccaagagcgcgaggtgccctgccacagaccttctccacacagcgacgaacaccaccatgatgacagcctgcctcatcctcagcaggccaccgacgatagcagcaaccagagcgacagcaacagcaacgagggcagacatctgctgctggtgtctggtgctggcgacggacctcctctgtgttctcaaaatcttggcgcccctggcggcggaccaaacaatggacctcaggaccccgacaacaccgacgacaatggccctcaagatcctgataataccgatgacaacggcccacacgaccctctgcctcaagacccagataacacagacgataacggtccacaagatccggacaatactgacgataatggaccccacgatccactgcctcacaaccctagcgatagcgccggaaatgatggcggacctccacagctgaccgaggaagtggaaaacaaaggcggagatcagggccctcctctgatgaccgatggcggaggtggacactctcacgattctggccacgacggcatcgaccctcatctgcctacactgctgctcggcacatctggctctggcggcgacgatgatgatcctcatggacctgtgcagctgagctactacgac

SEQ ID NO: 20 - protein, 898 aa, Artificial sequence
  Fusion of LMP1 of Epstein Barr virus and IPS1 of Homo sapieins
MDLDLERGPPGPRRPPRGPPLSSSIGLALLLLLLALLFWLYIIMSNWTGGALLVLYAFALMLVIIILIIFIFRRDLLCPLGALCLLLLMITLLLIALWNLHGQALYLGIVLFIFGCLLVLGLWIYLLEILWRLGATIWQLLAFFLAFFLDIILLIIALYLQQNWWTLLVDLLWLLLFLAILIWMYYHGQRPFAEDKTYKYICRNFSNFCNVDVVEILPYLPCLTARDQDRLRATCTLSGNRDTLWHLFNTLQRRPGWVEYFIAALRGCELVDLADEVASVYQSYQPRTSDRPPDPLEPPSLPAERPGPPTPAAAHSIPYNSCREKEPSYPMPVQETQAPESPGENSEQALQTLSPRAIPRNPDGGPLESSSDLAALSPLTSSGHQEQDTELGSTHTAGATSSLTPSRGPVSPSVSFQPLARSTPRASRLPGPTGSVVSTGTSFSSSSPGLASAGAAEGKQGAESDQAEPIICSSGAEAPANSLPSKVPTTLMPVNTVALKVPANPASVSTVPSKLPTSSKPPGAVPSNALTNPAPSKLPINSTRAGMVPSKVPTSMVLTKVSASTVPTDGSSRNEETPAAPTPAGATGGSSAWLDSSSENRGLGSELSKPGVLASQVDSPFSGCFEDLAISASTSLGMGPCHGPEENEYKSEGTFGIHVAENPSIQLLEGNPGPPADPDGGPRPQADRKFQEREVPCHRPSPHSDEHHHDDSLPHPQQATDDSSNQSDSNSNEGRHLLLVSGAGDGPPLCSQNLGAPGGGPNNGPQDPDNTDDNGPQDPDNTDDNGPHDPLPQDPDNTDDNGPQDPDNTDDNGPHDPLPHNPSDSAGNDGGPPQLTEEVENKGGDQGPPLMTDGGGGHSHDSGHDGIDPHLPTLLLGTSGSGGDDDDPHGPVQLSYYD

SEQ ID NO: 21 - DNA, 2541 bp, Artificial sequence
  Fusion of LMP1 of Epstein Barr virus and IPS1 of Homo sapiens
atggatctggatctcgaaagaggacctcctggacctagacggcctcctagaggaccacctctgagcagctctattggactggccctgctgctgcttctgctggctctgctgttctggctgtacatcatcatgagcaactggaccggcggagcactgctggtgctgtatgcctttgctctgatgctggtcatcatcatcctgatcatcttcatcttccggcgggacctgctgtgtcctctgggagcactttgtctgttgctgctgatgatcaccctcctgctgatcgccctgtggaacctgcatggacaggccctgtatctgggcatcgtgctgttcatcttcggctgcctgctggttctcggcctgtggatctacctgctggaaatcctttggagactgggcgccaccatctggcagctgctggcctttttcctggccttctttctggatatcatcctcctcatcattgccctgtacctgcagcagaactggtggaccctgctggtggatctgctttggctgctgctctttctggccatcctgatttggatgtactaccacggccagcggcctttcgccgaggacaagacctacaagtacatctgccggaacttcagcaacttctgcaacgtggacgtggtggaaattctgccctacctgccttgcctgaccgccagagatcaggacagactgagagccacatgtaccctgagcggcaacagagacacactgtggcacctgttcaacaccctgcagagaaggcctggctgggtcgagtactttatcgccgctctgagaggctgcgagctggtcgatctggctgatgaagtggccagcgtgtaccagagctaccagcctagaaccagcgaccggggcgagaatagcgaacaggctctgcagacactgagccccagagccattcctagaaaccctgatggcggccctctggaaagctctagtgatctggccgctctgtcccctctgacaagctctggacaccaagagcaggataccgagctgggcagcacacatacagccggcgctacaagcagcctgacaccttctagaggccccgtgtctcccagcgtgtcatttcagcctctggccaggtctacccctagggcttctagactgcctggaccaacaggcagcgtggtgtctaccggcacaagcttcagctctagctctcctggactggctagtgccggtgccgctgagggaaaacaaggcgccgaatctgatcaggccgagcctatcatctgtagcagcggagcagaagcccctgccaatagcctgcctagcaaggtgccaaccacactgatgcccgtgaacacagtggccctgaaggtgccagctaatcctgcctccgtgtccaccgtgccttctaagctgccaaccagctctaagccacctggcgccgtgccatctaacgccctgacaaatcctgctccaagcaagctgcccatcaactccacaagagccggcatggtgccctctaaggtgcccacatctatggtgctgaccaaggtgtccgccagcaccgtgccaacagatggcagctccagaaacgaggaaacccctgccgctcctactcctgctggcgctacaggcggatcttctgcttggctggatagcagcagcgagaacagaggcctgggcagcgagctttctaaacctggcgtgctggcttcccaggtggacagcccattttccggctgctttgaggacctggctatcagcgcctctacaagcctcggcatgggaccttgtcacggccccgaggaaaacgagtacaagagcgagggcaccttcggcatccacgtggccgagaatcctagcatccaactgctggaaggcaaccccggacctccagctgatccagatggcggaccaagacctcaggccgacagaaagttccaagagcgcgaggtgccctgccacagaccttctccacacagcgacgaacaccaccatgatgacagcctgcctcatcctcagcaggccaccgacgatagcagcaaccagagcgacagcaacagcaacgagggcagacatctgctgctggtgtctggtgctggcgacggacctcctctgtgttctcaaaatcttggcgcccctggcggcggaccaaacaatggacctcaggaccccgacaacaccgacgacaatggccctcaagatcctgataataccgatgacaacggcccacacgaccctctgcctcaagacccagataacacagacgataacggtccacaagatccggacaatactgacgataatggaccccacgatccactgcctcacaaccctagcgatagcgccggaaatgatggcggacctccacagctgaccgaggaagtggaaaacaaaggcggagatcagggccctcctctgatgaccgatggcggaggtggacactctcacgattctggccacgacggcatcgaccctcatctgcctacactgctgctcggcacatctggctctggcggcgacgatgatgatcctcatggacctgtgcagctgagctactacgac

SEQ ID NO: 22 - protein, 847 aa, Artificial sequence
  Fusion of LMP1 of Epstein Barr virus and IPS1 of Homo sapiens
MDLDLERGPPGPRRPPRGPPLSSSIGLALLLLLLALLFWLYIIMSNWTGGALLVLYAFALMLVIIILIIFIFRRDLLCPLGALCLLLLMITLLLIALWNLHGQALYLGIVLFIFGCLLVLGLWIYLLEILWRLGATIWQLLAFFLAFFLDIILLIIALYLQQNWWTLLVDLLWLLLFLAILIWMYYHGQRPFAEDKTYKYICRNFSNFCNVDVVEILPYLPCLTARDQDRLRATCTLSGNRDTLWHLFNTLQRRPGWVEYFIAALRGCELVDLADEVASVYQSYQPRTSDRGENSEQALQTLSPRAIPRNPDGGPLESSSDLAALSPLTSSGHQEQDTELGSTHTAGATSSLTPSRGPVSPSVSFQPLARSTPRASRLPGPTGSVVSTGTSFSSSSPGLASAGAAEGKQGAESDQAEPIICSSGAEAPANSLPSKVPTTLMPVNTVALKVPANPASVSTVPSKLPTSSKPPGAVPSNALTNPAPSKLPINSTRAGMVPSKVPTSMVLTKVSASTVPTDGSSRNEETPAAPTPAGATGGSSAWLDSSSENRGLGSELSKPGVLASQVDSPFSGCFEDLAISASTSLGMGPCHGPEENEYKSEGTFGIHVAENPSIQLLEGNPGPPADPDGGPRPQADRKFQEREVPCHRPSPHSDEHHHDDSLPHPQQATDDSSNQSDSNSNEGRHLLLVSGAGDGPPLCSQNLGAPGGGPNNGPQDPDNTDDNGPQDPDNTDDNGPHDPLPQDPDNTDDNGPQDPDNTDDNGPHDPLPHNPSDSAGNDGGPPQLTEEVENKGGDQGPPLMTDGGGGHSHDSGHDGIDPHLPTLLLGTSGSGGDDDDPHGPVQLSYYD

SEQ ID NO: 23 - DNA, 2697 bp, Artificial sequence
  Fusion of LMP1 of Epstein Barr virus and IPS1 of Homo sapiens
atggatctggatctcgaaagaggacctcctggacctagacggcctcctagaggaccacctctgagcagctctattggactggccctgctgctgcttctgctggctctgctgttctggctgtacatcatcatgagcaactggaccggcggagcactgctggtgctgtatgcctttgctctgatgctggtcatcatcatcctgatcatcttcatcttccggcgggacctgctgtgtcctctgggagcactttgtctgttgctgctgatgatcaccctcctgctgatcgccctgtggaacctgcatggacaggccctgtatctgggcatcgtgctgttcatcttcggctgcctgctggttctcggcctgtggatctacctgctggaaatcctttggagactgggcgccaccatctggcagctgctggcctttttcctggccttctttctggatatcatcctcctcatcattgccctgtacctgcagcagaactggtggaccctgctggtggatctgctttggctgctgctctttctggccatcctgatttggatgtactaccacggccagcggccttctccaagacactgcccagtggaaagagagcagttcaagagggacgcccagcctagacctggcggagatcctgatgctccacctggaccaaatggcgagctgctgcagatcagccctaatgaggccgtgcacatcggcttcaccggcgagtctaagtacgagaacgaggaacccggccactgtcctggcatgggcctttctacatctgcctctatcgccctggacgagttctgcggcagctttccatctgatgtgcagtctgccctcgtgggccctaagtctctggaatctggcctgggcagaaacgagagcagctccgatctgtgggctagctctggtggaacagctggcgctcctacaccagccgctcctaccgaagagaatagaagcagcggcgacacccctgtgacaagcgcctctgtgaaaaccctggtcatgagcaccccagtgaagtccccagtgatgggcgccagaacctccaacattcccctgaagtctcccgctcctaacacactggccaactctccagtggctggccctcctaagtctagcacccctctgaaaagccccgtgacctctgtgtctgcccctaacgctcctgtgaaactggccgtgaccaacgtgcccatgctgaccacacctgtgaaatccccactgagcaatgcccctgccgaggccggaagctcttgtatcattcccgaggctcaggatagcgaggctggccaaaaaggcgaagctgcaggcgcttctgctctgggccctagctctagctcttttagcaccggcaccagcgtggtgtctggcacaccaggacctctgagaagcgccagacctacctctagagccctgcctcagtttagcgtgtcccctagtgtgcctggcagaagccctacactgtctagtacagccggcgctacacacaccagcggactggaaacagaccaagaacagcatggcagcagcaccctgccttctctggctgcccttgattctagcagcgaactgccaggcggcgaccccaatagacctatcgctagacctagcctgacacagctggcccaagagagcaatgagggcccttctgagcctgctcagaccgaacaggtgccaatgccttacagccccgagaaagagcggtgcagcaactaccctatcagccatgccgctgctcccacacctcctggtccaagagaagctcctctgagccctcctgagctgcccgatcctccaagagatagcaccagacctcagtactcccagtacgtgtccgccgtggaagatgccctggatgtgctggaatgtggcagactggccgccatcttctacgaagtgtggggccctagaaggcagctgaccaactttctgcactggctgaccgacagaaacggcagcctgacatgtaccgccagactgagagatcaggaccgggccacactgtgccctctgtatcctctgatcgaggtggtggacgtgaactgcttcaacagcttcaaccggtgcatctacaagtacaccaaggacgaggctttccctatgcacagcgacgaacaccaccatgatgacagcctgcctcatcctcagcaggccaccgacgatagcagcaaccagagcgacagcaacagcaacgagggcagacatctgctgctggtgtctggtgctggcgacggacctcctctgtgttctcaaaatcttggcgcccctggcggcggaccaaacaatggacctcaggaccccgacaacaccgacgacaatggccctcaagatcctgataataccgatgacaacggcccacacgaccctctgcctcaagacccagataacacagacgataacggtccacaagatccggacaatactgacgataatggaccccacgatccactgcctcacaaccctagcgatagcgccggaaatgatggcggacctccacagctgaccgaggaagtggaaaacaaaggcggagatcagggccctcctctgatgaccgatggcggaggtggacactctcacgattctggccacgacggcatcgaccctcatctgcctacactgctgctcggcacatctggctctggcggcgacgatgatgatcctcatggacctgtgcagctgagctactacgac

SEQ ID NO: 24 - protein, 899 aa, Artificial sequence
  Fusion of LMP1 of Epstein Barr virus and IPS1 of Homo sapiens
MDLDLERGPPGPRRPPRGPPLSSSIGLALLLLLLALLFWLYIIMSNWTGGALLVLYAFALMLVIIILIIFIFRRDLLCPLGALCLLLLMITLLLIALWNLHGQALYLGIVLFIFGCLLVLGLWIYLLEILWRLGATIWQLLAFFLAFFLDIILLIIALYLQQNWWTLLVDLLWLLLFLAILIWMYYHGQRPSPRHCPVEREQFKRDAQPRPGGDPDAPPGPNGELLQISPNEAVHIGFTGESKYENEEPGHCPGMGLSTSASIALDEFCGSFPSDVQSALVGPKSLESGLGRNESSSDLWASSGGTAGAPTPAAPTEENRSSGDTPVTSASVKTLVMSTPVKSPVMGARTSNIPLKSPAPNTLANSPVAGPPKSSTPLKSPVTSVSAPNAPVKLAVTNVPMLTTPVKSPLSNAPAEAGSSCIIPEAQDSEAGQKGEAAGASALGPSSSSFSTGTSVVSGTPGPLRSARPTSRALPQFSVSPSVPGRSPTLSSTAGATHTSGLETDQEQHGSSTLPSLAALDSSSELPGGDPNRPIARPSLTQLAQESNEGPSEPAQTEQVPMPYSPEKERCSNYPISHAAAPTPPGPREAPLSPPELPDPPRDSTRPQYSQYVSAVEDALDVLECGRLAAIFYEVWGPRRQLTNFLHWLTDRNGSLTCTARLRDQDRATLCPLYPLIEVVDVNCFNSFNRCIYKYTKDEAFPMHSDEHHHDDSLPHPQQATDDSSNQSDSNSNEGRHLLLVSGAGDGPPLCSQNLGAPGGGPNNGPQDPDNTDDNGPQDPDNTDDNGPHDPLPQDPDNTDDNGPQDPDNTDDNGPHDPLPHNPSDSAGNDGGPPQLTEEVENKGGDQGPPLMTDGGGGHSHDSGHDGIDPHLPTLLLGTSGSGGDDDDPHGPVQLSYYD